European Patent Specification EP 3 429 543 B1, published November 20, 2024. Title: SELECTIVELY VENTED BIOLOGICAL ASSAY DEVICES AND ASSOCIATED METHODS. Applicant: DIASSESS INC. Application PCT/US2017/022306. The sequence listing filed with the application follows.

SEQUENCE LISTING (5 sequences)

SEQ ID NO: 1 - DNA, 20 bp, Artificial Sequence
  Description of Artificial Sequence: Synthetic primer
gatctgaatccgaccaaccg

SEQ ID NO: 2 - DNA, 18 bp, Artificial Sequence
  Description of Artificial Sequence: Synthetic primer
aacgcccacgctctcgca

SEQ ID NO: 3 - DNA, 41 bp, Artificial Sequence
  Description of Artificial Sequence: Synthetic primer
aaatccgtccagtggtttttttgaaaatcgttgtatctccg

SEQ ID NO: 4 - DNA, 46 bp, Artificial Sequence
  Description of Artificial Sequence: Synthetic primer
ccgaaaccactggacggatttttatttttaatctaaaacaaacatc

SEQ ID NO: 5 - DNA, 121 bp, Schistosoma mansoni
gatctgaatccgaccaaccgttctatgaaaatcgttgtatctccgaaaccactggacggatttttatgatgtttgttttagattatttgcgagagcgtgggcgttaatataaaacaagaat